European Patent Application EP 4 471 068 A1, published December 4, 2024. Title: 一种PD1抗体与白介素2融合的双功能分子. Applicant: 中国科学院生物物理研究所. The sequence listing filed with the application follows.

SEQUENCE LISTING (23 sequences)

SEQ ID NO: 1 - protein, 133 aa, Homo sapiens [sequence omitted]

SEQ ID NO: 2 - protein, 227 aa, Homo sapiens
DKTHTCPPCPAPELLGGPSVFLFPPKPKDTLMISRTPEVTCVVVDVSHEDPEVKFNWYVDGVEVHNAKTKPREEQYNSTYRVVSVLTVLHQDWLNGKEYKCKVSNKALPAPIEKTISKAKGQPREPQVYTLPPSRDELTKNQVSLTCLVKGFYPSDIAVEWESNGQPENNYKTTPPVLDSDGSFFLYSKLTVDKSRWQQGNVFSCSVMHEALHNHYTQKSLSLSPGK

SEQ ID NO: 3 - protein, 227 aa, Artificial sequence
DKTHTCPPCPAPEAAGGPSVFLFPPKPKDTLMISRTPEVTCVVVDVSHEDPEVKFNWYVDGVEVHNAKTKPREEQYNSTYRVVSVLTVLHQDWLNGKEYKCKVSNKALGAPIEKTISKAKGQPREPQVYTLPPSRDELTKNQVSLTCLVKGFYPSDIAVEWESNGQPENNYKTTPPVLDSDGSFFLYSKLTVDKSRWQQGNVFSCSVMHEALHNHYTQKSLSLSPGK

SEQ ID NO: 4 - protein, 227 aa, Artificial sequence
DKTHTCPPCPAPELLGGPSVFLFPPKPKDTLMISRTPEVTCVVVDVSHEDPEVKFNWYVDGVEVHNAKTKPREEQYNSTYRVVSVLTVLHQDWLNGKEYKCKVSNKALPAPIEKTISKAKGQPREPQVCTLPPSRDELTKNQVSLSCAVKGFYPSDIAVEWESNGQPENNYKTTPPVLDSDGSFKLVSKLTVDKSRWQQGNVFSCSVMHEALHNHYTQKSLSLSPGK

SEQ ID NO: 5 - protein, 227 aa, Artificial sequence
DKTHTCPPCPAPELLGGPSVFLFPPKPKDTLMISRTPEVTCVVVDVSHEDPEVKFNWYVDGVEVHNAKTKPREEQYNSTYRVVSVLTVLHQDWLNGKEYKCKVSNKALPAPIEKTISKAKGQPREPQVYTLPPCRDELTKNQVSLWCLVKGFYPSDIAVEWESNGQPENNYKTTPPVLDSDGSFFLYSALTVDKSRWQQGNVFSCSVMHEALHNHYTQKSLSLSPGK

SEQ ID NO: 6 - protein, 5 aa, Artificial sequence
GGGGS

SEQ ID NO: 7 - protein, 214 aa, Artificial sequence
EIVLTQSPATLSLSPGERATLSCRASQSVSSYLAWYQQKPGQAPRLLIYDASNRATGIPARFSGSGSGTDFTLTISSLEPEDFAVYYCQQSSNWPRTFGQGTKVEIKRTVAAPSVFIFPPSDEQLKSGTASVVCLLNNFYPREAKVQWKVDNALQSGNSQESVTEQDSKDSTYSLSSTLTLSKADYEKHKVYACEVTHQGLSSPVTKSFNRGEC

SEQ ID NO: 8 - protein, 648 aa, Artificial sequence
GLNVALGLNLEUVALGLUSERGLYGLYGLYVALVALGLNPROGLYARGSERLEUARGLEUASPCYSLYSALASERGLYILETHRPHESERASNSERGLYMETHISTRPVALARGGLNALAPROGLYLYSGLYLEUGLUTRPVALALAVALILETRPTYRASPGLYSERLYSARGTYRTYRALAASPSERVALLYSGLYARGPHETHRILESERARGASPASNSERLYSASNTHRLEUPHELEUGLNMETASNSERLEUARGALAGLUASPTHRALAVALTYRTYRCYSALATHRASNASPASPTYRTRPGLYGLNGLYTHRLEUVALTHRVALSERSERALASERTHRLYSGLYPROSERVALPHEPROLEUALAPROSERSERLYSSERTHRSERGLYGLYTHRALAALALEUGLYCYSLEUVALLYSASPTYRPHEPROGLUPROVALTHRVALSERTRPASNSERGLYALALEUTHRSERGLYVALHISTHRPHEPROALAVALLEUGLNSERSERGLYLEUTYRSERLEUSERSERVALVALTHRVALPROSERSERSERLEUGLYTHRGLNTHRTYRILECYSASNVALASNHISLYSPROSERASNTHRLYSVALASPLYSARGVALGLUPROLYSSERCYS

SEQ ID NO: 9 - protein, 705 aa, Artificial sequence
GLUILEVALLEUTHRGLNSERPROALATHRLEUSERLEUSERPROGLYGLUARGALATHRLEUSERCYSARGALASERGLNSERVALSERSERTYRLEUALATRPTYRGLNGLNLYSPROGLYGLNALAPROARGLEULEUILETYRASPALASERASNARGALATHRGLYILEPROALAARGPHESERGLYSERGLYSERGLYTHRASPPHETHRLEUTHRILESERSERLEUGLUPROGLUASPPHEALAVALTYRTYRCYSGLNGLNSERSERASNTRPPROARGTHRPHEGLYGLNGLYTHRLYSVALGLUILELYSGLYGLYGLYGLYSERGLYGLYGLYGLYSERGLYGLYGLYGLYSERGLNVALGLNLEUVALGLUSERGLYGLYGLYVALVALGLNPROGLYARGSERLEUARGLEUASPCYSLYSALASERGLYILETHRPHESERASNSERGLYMETHISTRPVALARGGLNALAPROGLYLYSGLYLEUGLUTRPVALALAVALILETRPTYRASPGLYSERLYSARGTYRTYRALAASPSERVALLYSGLYARGPHETHRILESERARGASPASNSERLYSASNTHRLEUPHELEUGLNMETASNSERLEUARGALAGLUASPTHRALAVALTYRTYRCYSALATHRASNASPASPTYRTRPGLYGLNGLYTHRLEUVALTHRVALSERSER

SEQ ID NO: 10 - protein, 1095 aa, Artificial sequence
ALAPROTHRSERSERSERTHRLYSLYSTHRGLNLEUGLNLEUGLUHISLEULEULEUASPLEUGLNMETILELEUASNGLYILEASNASNTYRLYSASNPROLYSLEUTHRLEUMETLEUTHRALALYSPHETYRMETPROLYSLYSALATHRGLULEULYSHISLEUGLNCYSLEUGLUGLUGLULEULYSPROLEUGLUGLUVALLEUASNLEUALAGLNSERLYSASNPHEHISLEUARGPROARGASPLEUILESERASNILEASNVALILEVALLEUGLULEULYSGLYSERGLUTHRTHRPHEMETCYSGLUTYRALAASPGLUTHRALATHRILEVALGLUPHELEUASNARGTRPILETHRPHECYSGLNSERILEILESERTHRLEUTHRGLYGLYGLYGLYSERASPLYSTHRHISTHRCYSPROPROCYSPROALAPROGLULEULEUGLYGLYPROSERVALPHELEUPHEPROPROLYSPROLYSASPTHRLEUMETILESERARGTHRPROGLUVALTHRCYSVALVALVALASPVALSERHISGLUASPPROGLUVALLYSPHEASNTRPTYRVALASPGLYVALGLUVALHISASNALALYSTHRLYSPROARGGLUGLUGLNTYRASNSERTHRTYRARGVALVALSERVALLEUTHRVALLEUHISGLNASPTRPLEUASNGLYLYSGLUTYRLYSCYSLYSVALSERASNLYSALALEUPROALAPROILEGLULYSTHRILESERLYSALALYSGLYGLNPROARGGLUPROGLNVALCYSTHRLEUPROPROSERARGASPGLULEUTHRLYSASNGLNVALSERLEUSERCYSALAVALLYSGLYPHETYRPROSERASPILEALAVALGLUTRPGLUSERASNGLYGLNPROGLUASNASNTYRLYSTHRTHRPROPROVALLEUASPSERASPGLYSERPHELYSLEUVALSERLYSLEUTHRVALASPLYSSERARGTRPGLNGLNGLYASNVALPHESERCYSSERVALMETHISGLUALALEUHISASNHISTYRTHRGLNLYSSERLEUSERLEUSERPROGLYLYS

SEQ ID NO: 11 - protein, 1329 aa, Artificial sequence
GLNVALGLNLEUVALGLUSERGLYGLYGLYVALVALGLNPROGLYARGSERLEUARGLEUASPCYSLYSALASERGLYILETHRPHESERASNSERGLYMETHISTRPVALARGGLNALAPROGLYLYSGLYLEUGLUTRPVALALAVALILETRPTYRASPGLYSERLYSARGTYRTYRALAASPSERVALLYSGLYARGPHETHRILESERARGASPASNSERLYSASNTHRLEUPHELEUGLNMETASNSERLEUARGALAGLUASPTHRALAVALTYRTYRCYSALATHRASNASPASPTYRTRPGLYGLNGLYTHRLEUVALTHRVALSERSERALASERTHRLYSGLYPROSERVALPHEPROLEUALAPROSERSERLYSSERTHRSERGLYGLYTHRALAALALEUGLYCYSLEUVALLYSASPTYRPHEPROGLUPROVALTHRVALSERTRPASNSERGLYALALEUTHRSERGLYVALHISTHRPHEPROALAVALLEUGLNSERSERGLYLEUTYRSERLEUSERSERVALVALTHRVALPROSERSERSERLEUGLYTHRGLNTHRTYRILECYSASNVALASNHISLYSPROSERASNTHRLYSVALASPLYSARGVALGLUPROLYSSERCYSASPLYSTHRHISTHRCYSPROPROCYSPROALAPROGLULEULEUGLYGLYPROSERVALPHELEUPHEPROPROLYSPROLYSASPTHRLEUMETILESERARGTHRPROGLUVALTHRCYSVALVALVALASPVALSERHISGLUASPPROGLUVALLYSPHEASNTRPTYRVALASPGLYVALGLUVALHISASNALALYSTHRLYSPROARGGLUGLUGLNTYRASNSERTHRTYRARGVALVALSERVALLEUTHRVALLEUHISGLNASPTRPLEUASNGLYLYSGLUTYRLYSCYSLYSVALSERASNLYSALALEUPROALAPROILEGLULYSTHRILESERLYSALALYSGLYGLNPROARGGLUPROGLNVALTYRTHRLEUPROPROCYSARGASPGLULEUTHRLYSASNGLNVALSERLEUTRPCYSLEUVALLYSGLYPHETYRPROSERASPILEALAVALGLUTRPGLUSERASNGLYGLNPROGLUASNASNTYRLYSTHRTHRPROPROVALLEUASPSERASPGLYSERPHEPHELEUTYRSERALALEUTHRVALASPLYSSERARGTRPGLNGLNGLYASNVALPHESERCYSSERVALMETHISGLUALALEUHISASNHISTYRTHRGLNLYSSERLEUSERLEUSERPROGLYLYS

SEQ ID NO: 12 - protein, 1386 aa, Artificial sequence
GLUILEVALLEUTHRGLNSERPROALATHRLEUSERLEUSERPROGLYGLUARGALATHRLEUSERCYSARGALASERGLNSERVALSERSERTYRLEUALATRPTYRGLNGLNLYSPROGLYGLNALAPROARGLEULEUILETYRASPALASERASNARGALATHRGLYILEPROALAARGPHESERGLYSERGLYSERGLYTHRASPPHETHRLEUTHRILESERSERLEUGLUPROGLUASPPHEALAVALTYRTYRCYSGLNGLNSERSERASNTRPPROARGTHRPHEGLYGLNGLYTHRLYSVALGLUILELYSGLYGLYGLYGLYSERGLYGLYGLYGLYSERGLYGLYGLYGLYSERGLNVALGLNLEUVALGLUSERGLYGLYGLYVALVALGLNPROGLYARGSERLEUARGLEUASPCYSLYSALASERGLYILETHRPHESERASNSERGLYMETHISTRPVALARGGLNALAPROGLYLYSGLYLEUGLUTRPVALALAVALILETRPTYRASPGLYSERLYSARGTYRTYRALAASPSERVALLYSGLYARGPHETHRILESERARGASPASNSERLYSASNTHRLEUPHELEUGLNMETASNSERLEUARGALAGLUASPTHRALAVALTYRTYRCYSALATHRASNASPASPTYRTRPGLYGLNGLYTHRLEUVALTHRVALSERSERASPLYSTHRHISTHRCYSPROPROCYSPROALAPROGLULEULEUGLYGLYPROSERVALPHELEUPHEPROPROLYSPROLYSASPTHRLEUMETILESERARGTHRPROGLUVALTHRCYSVALVALVALASPVALSERHISGLUASPPROGLUVALLYSPHEASNTRPTYRVALASPGLYVALGLUVALHISASNALALYSTHRLYSPROARGGLUGLUGLNTYRASNSERTHRTYRARGVALVALSERVALLEUTHRVALLEUHISGLNASPTRPLEUASNGLYLYSGLUTYRLYSCYSLYSVALSERASNLYSALALEUPROALAPROILEGLULYSTHRILESERLYSALALYSGLYGLNPROARGGLUPROGLNVALTYRTHRLEUPROPROCYSARGASPGLULEUTHRLYSASNGLNVALSERLEUTRPCYSLEUVALLYSGLYPHETYRPROSERASPILEALAVALGLUTRPGLUSERASNGLYGLNPROGLUASNASNTYRLYSTHRTHRPROPROVALLEUASPSERASPGLYSERPHEPHELEUTYRSERALALEUTHRVALASPLYSSERARGTRPGLNGLNGLYASNVALPHESERCYSSERVALMETHISGLUALALEUHISASNHISTYRTHRGLNLYSSERLEUSERLEUSERPROGLYLYS

SEQ ID NO: 13 - protein, 218 aa, Artificial sequence
EIVLTQSPATLSLSPGERATLSCRASKGVSTSGYSYLHWYQQKPGQAPRLLIYLASYLESGVPARFSGSGSGTDFTLTISSLEPEDFAVYYCQHSRDLPLTFGGGTKVEIKRTVAAPSVFIFPPSDEQLKSGTASVVCLLNNFYPREAKVQWKVDNALQSGNSQESVTEQDSKDSTYSLSSTLTLSKADYEKHKVYACEVTHQGLSSPVTKSFNRGEC

SEQ ID NO: 14 - protein, 669 aa, Artificial sequence
GLNVALGLNLEUVALGLNSERGLYVALGLUVALLYSLYSPROGLYALASERVALLYSVALSERCYSLYSALASERGLYTYRTHRPHETHRASNTYRTYRMETTYRTRPVALARGGLNALAPROGLYGLNGLYLEUGLUTRPMETGLYGLYILEASNPROSERASNGLYGLYTHRASNPHEASNGLULYSPHELYSASNARGVALTHRLEUTHRTHRASPSERSERTHRTHRTHRALATYRMETGLULEULYSSERLEUGLNPHEASPASPTHRALAVALTYRTYRCYSALAARGARGASPTYRARGPHEASPMETGLYPHEASPTYRTRPGLYGLNGLYTHRTHRVALTHRVALSERSERALASERTHRLYSGLYPROSERVALPHEPROLEUALAPROSERSERLYSSERTHRSERGLYGLYTHRALAALALEUGLYCYSLEUVALLYSASPTYRPHEPROGLUPROVALTHRVALSERTRPASNSERGLYALALEUTHRSERGLYVALHISTHRPHEPROALAVALLEUGLNSERSERGLYLEUTYRSERLEUSERSERVALVALTHRVALPROSERSERSERLEUGLYTHRGLNTHRTYRILECYSASNVALASNHISLYSPROSERASNTHRLYSVALASPLYSARGVALGLUPROLYSSERCYS

SEQ ID NO: 15 - protein, 738 aa, Artificial sequence
GLUILEVALLEUTHRGLNSERPROALATHRLEUSERLEUSERPROGLYGLUARGALATHRLEUSERCYSARGALASERLYSGLYVALSERTHRSERGLYTYRSERTYRLEUHISTRPTYRGLNGLNLYSPROGLYGLNALAPROARGLEULEUILETYRLEUALASERTYRLEUGLUSERGLYVALPROALAARGPHESERGLYSERGLYSERGLYTHRASPPHETHRLEUTHRILESERSERLEUGLUPROGLUASPPHEALAVALTYRTYRCYSGLNHISSERARGASPLEUPROLEUTHRPHEGLYGLYGLYTHRLYSVALGLUILELYSGLYGLYGLYGLYSERGLYGLYGLYGLYSERGLYGLYGLYGLYSERGLNVALGLNLEUVALGLNSERGLYVALGLUVALLYSLYSPROGLYALASERVALLYSVALSERCYSLYSALASERGLYTYRTHRPHETHRASNTYRTYRMETTYRTRPVALARGGLNALAPROGLYGLNGLYLEUGLUTRPMETGLYGLYILEASNPROSERASNGLYGLYTHRASNPHEASNGLULYSPHELYSASNARGVALTHRLEUTHRTHRASPSERSERTHRTHRTHRALATYRMETGLULEULYSSERLEUGLNPHEASPASPTHRALAVALTYRTYRCYSALAARGARGASPTYRARGPHEASPMETGLYPHEASPTYRTRPGLYGLNGLYTHRTHRVALTHRVALSERSER

SEQ ID NO: 16 - protein, 1350 aa, Artificial sequence
GLNVALGLNLEUVALGLNSERGLYVALGLUVALLYSLYSPROGLYALASERVALLYSVALSERCYSLYSALASERGLYTYRTHRPHETHRASNTYRTYRMETTYRTRPVALARGGLNALAPROGLYGLNGLYLEUGLUTRPMETGLYGLYILEASNPROSERASNGLYGLYTHRASNPHEASNGLULYSPHELYSASNARGVALTHRLEUTHRTHRASPSERSERTHRTHRTHRALATYRMETGLULEULYSSERLEUGLNPHEASPASPTHRALAVALTYRTYRCYSALAARGARGASPTYRARGPHEASPMETGLYPHEASPTYRTRPGLYGLNGLYTHRTHRVALTHRVALSERSERALASERTHRLYSGLYPROSERVALPHEPROLEUALAPROSERSERLYSSERTHRSERGLYGLYTHRALAALALEUGLYCYSLEUVALLYSASPTYRPHEPROGLUPROVALTHRVALSERTRPASNSERGLYALALEUTHRSERGLYVALHISTHRPHEPROALAVALLEUGLNSERSERGLYLEUTYRSERLEUSERSERVALVALTHRVALPROSERSERSERLEUGLYTHRGLNTHRTYRILECYSASNVALASNHISLYSPROSERASNTHRLYSVALASPLYSARGVALGLUPROLYSSERCYSASPLYSTHRHISTHRCYSPROPROCYSPROALAPROGLULEULEUGLYGLYPROSERVALPHELEUPHEPROPROLYSPROLYSASPTHRLEUMETILESERARGTHRPROGLUVALTHRCYSVALVALVALASPVALSERHISGLUASPPROGLUVALLYSPHEASNTRPTYRVALASPGLYVALGLUVALHISASNALALYSTHRLYSPROARGGLUGLUGLNTYRASNSERTHRTYRARGVALVALSERVALLEUTHRVALLEUHISGLNASPTRPLEUASNGLYLYSGLUTYRLYSCYSLYSVALSERASNLYSALALEUPROALAPROILEGLULYSTHRILESERLYSALALYSGLYGLNPROARGGLUPROGLNVALTYRTHRLEUPROPROCYSARGASPGLULEUTHRLYSASNGLNVALSERLEUTRPCYSLEUVALLYSGLYPHETYRPROSERASPILEALAVALGLUTRPGLUSERASNGLYGLNPROGLUASNASNTYRLYSTHRTHRPROPROVALLEUASPSERASPGLYSERPHEPHELEUTYRSERALALEUTHRVALASPLYSSERARGTRPGLNGLNGLYASNVALPHESERCYSSERVALMETHISGLUALALEUHISASNHISTYRTHRGLNLYSSERLEUSERLEUSERPROGLYLYS

SEQ ID NO: 17 - protein, 1419 aa, Artificial sequence
GLUILEVALLEUTHRGLNSERPROALATHRLEUSERLEUSERPROGLYGLUARGALATHRLEUSERCYSARGALASERLYSGLYVALSERTHRSERGLYTYRSERTYRLEUHISTRPTYRGLNGLNLYSPROGLYGLNALAPROARGLEULEUILETYRLEUALASERTYRLEUGLUSERGLYVALPROALAARGPHESERGLYSERGLYSERGLYTHRASPPHETHRLEUTHRILESERSERLEUGLUPROGLUASPPHEALAVALTYRTYRCYSGLNHISSERARGASPLEUPROLEUTHRPHEGLYGLYGLYTHRLYSVALGLUILELYSGLYGLYGLYGLYSERGLYGLYGLYGLYSERGLYGLYGLYGLYSERGLNVALGLNLEUVALGLNSERGLYVALGLUVALLYSLYSPROGLYALASERVALLYSVALSERCYSLYSALASERGLYTYRTHRPHETHRASNTYRTYRMETTYRTRPVALARGGLNALAPROGLYGLNGLYLEUGLUTRPMETGLYGLYILEASNPROSERASNGLYGLYTHRASNPHEASNGLULYSPHELYSASNARGVALTHRLEUTHRTHRASPSERSERTHRTHRTHRALATYRMETGLULEULYSSERLEUGLNPHEASPASPTHRALAVALTYRTYRCYSALAARGARGASPTYRARGPHEASPMETGLYPHEASPTYRTRPGLYGLNGLYTHRTHRVALTHRVALSERSERASPLYSTHRHISTHRCYSPROPROCYSPROALAPROGLULEULEUGLYGLYPROSERVALPHELEUPHEPROPROLYSPROLYSASPTHRLEUMETILESERARGTHRPROGLUVALTHRCYSVALVALVALASPVALSERHISGLUASPPROGLUVALLYSPHEASNTRPTYRVALASPGLYVALGLUVALHISASNALALYSTHRLYSPROARGGLUGLUGLNTYRASNSERTHRTYRARGVALVALSERVALLEUTHRVALLEUHISGLNASPTRPLEUASNGLYLYSGLUTYRLYSCYSLYSVALSERASNLYSALALEUPROALAPROILEGLULYSTHRILESERLYSALALYSGLYGLNPROARGGLUPROGLNVALTYRTHRLEUPROPROCYSARGASPGLULEUTHRLYSASNGLNVALSERLEUTRPCYSLEUVALLYSGLYPHETYRPROSERASPILEALAVALGLUTRPGLUSERASNGLYGLNPROGLUASNASNTYRLYSTHRTHRPROPROVALLEUASPSERASPGLYSERPHEPHELEUTYRSERALALEUTHRVALASPLYSSERARGTRPGLNGLNGLYASNVALPHESERCYSSERVALMETHISGLUALALEUHISASNHISTYRTHRGLNLYSSERLEUSERLEUSERPROGLYLYS

SEQ ID NO: 18 - protein, 1800 aa, Artificial sequence
GLUILEVALLEUTHRGLNSERPROALATHRLEUSERLEUSERPROGLYGLUARGALATHRLEUSERCYSARGALASERGLNSERVALSERSERTYRLEUALATRPTYRGLNGLNLYSPROGLYGLNALAPROARGLEULEUILETYRASPALASERASNARGALATHRGLYILEPROALAARGPHESERGLYSERGLYSERGLYTHRASPPHETHRLEUTHRILESERSERLEUGLUPROGLUASPPHEALAVALTYRTYRCYSGLNGLNSERSERASNTRPPROARGTHRPHEGLYGLNGLYTHRLYSVALGLUILELYSGLYGLYGLYGLYSERGLYGLYGLYGLYSERGLYGLYGLYGLYSERGLNVALGLNLEUVALGLUSERGLYGLYGLYVALVALGLNPROGLYARGSERLEUARGLEUASPCYSLYSALASERGLYILETHRPHESERASNSERGLYMETHISTRPVALARGGLNALAPROGLYLYSGLYLEUGLUTRPVALALAVALILETRPTYRASPGLYSERLYSARGTYRTYRALAASPSERVALLYSGLYARGPHETHRILESERARGASPASNSERLYSASNTHRLEUPHELEUGLNMETASNSERLEUARGALAGLUASPTHRALAVALTYRTYRCYSALATHRASNASPASPTYRTRPGLYGLNGLYTHRLEUVALTHRVALSERSERASPLYSTHRHISTHRCYSPROPROCYSPROALAPROGLULEULEUGLYGLYPROSERVALPHELEUPHEPROPROLYSPROLYSASPTHRLEUMETILESERARGTHRPROGLUVALTHRCYSVALVALVALASPVALSERHISGLUASPPROGLUVALLYSPHEASNTRPTYRVALASPGLYVALGLUVALHISASNALALYSTHRLYSPROARGGLUGLUGLNTYRASNSERTHRTYRARGVALVALSERVALLEUTHRVALLEUHISGLNASPTRPLEUASNGLYLYSGLUTYRLYSCYSLYSVALSERASNLYSALALEUPROALAPROILEGLULYSTHRILESERLYSALALYSGLYGLNPROARGGLUPROGLNVALTYRTHRLEUPROPROSERARGASPGLULEUTHRLYSASNGLNVALSERLEUTHRCYSLEUVALLYSGLYPHETYRPROSERASPILEALAVALGLUTRPGLUSERASNGLYGLNPROGLUASNASNTYRLYSTHRTHRPROPROVALLEUASPSERASPGLYSERPHEPHELEUTYRSERLYSLEUTHRVALASPLYSSERARGTRPGLNGLNGLYASNVALPHESERCYSSERVALMETHISGLUALALEUHISASNHISTYRTHRGLNLYSSERLEUSERLEUSERPROGLYLYSGLYGLYGLYGLYSERALAPROTHRSERSERSERTHRLYSLYSTHRGLNLEUGLNLEUGLUHISLEULEULEUASPLEUGLNMETILELEUASNGLYILEASNASNTYRLYSASNPROLYSLEUTHRLEUMETLEUTHRALALYSPHETYRMETPROLYSLYSALATHRGLULEULYSHISLEUGLNCYSLEUGLUGLUGLULEULYSPROLEUGLUGLUVALLEUASNLEUALAGLNSERLYSASNPHEHISLEUARGPROARGASPLEUILESERASNILEASNVALILEVALLEUGLULEULYSGLYSERGLUTHRTHRPHEMETCYSGLUTYRALAASPGLUTHRALATHRILEVALGLUPHELEUASNARGTRPILETHRPHECYSGLNSERILEILESERTHRLEUTHR

SEQ ID NO: 19 - protein, 1800 aa, Artificial sequence
ALAPROTHRSERSERSERTHRLYSLYSTHRGLNLEUGLNLEUGLUHISLEULEULEUASPLEUGLNMETILELEUASNGLYILEASNASNTYRLYSASNPROLYSLEUTHRLEUMETLEUTHRALALYSPHETYRMETPROLYSLYSALATHRGLULEULYSHISLEUGLNCYSLEUGLUGLUGLULEULYSPROLEUGLUGLUVALLEUASNLEUALAGLNSERLYSASNPHEHISLEUARGPROARGASPLEUILESERASNILEASNVALILEVALLEUGLULEULYSGLYSERGLUTHRTHRPHEMETCYSGLUTYRALAASPGLUTHRALATHRILEVALGLUPHELEUASNARGTRPILETHRPHECYSGLNSERILEILESERTHRLEUTHRGLYGLYGLYGLYSERGLUILEVALLEUTHRGLNSERPROALATHRLEUSERLEUSERPROGLYGLUARGALATHRLEUSERCYSARGALASERGLNSERVALSERSERTYRLEUALATRPTYRGLNGLNLYSPROGLYGLNALAPROARGLEULEUILETYRASPALASERASNARGALATHRGLYILEPROALAARGPHESERGLYSERGLYSERGLYTHRASPPHETHRLEUTHRILESERSERLEUGLUPROGLUASPPHEALAVALTYRTYRCYSGLNGLNSERSERASNTRPPROARGTHRPHEGLYGLNGLYTHRLYSVALGLUILELYSGLYGLYGLYGLYSERGLYGLYGLYGLYSERGLYGLYGLYGLYSERGLNVALGLNLEUVALGLUSERGLYGLYGLYVALVALGLNPROGLYARGSERLEUARGLEUASPCYSLYSALASERGLYILETHRPHESERASNSERGLYMETHISTRPVALARGGLNALAPROGLYLYSGLYLEUGLUTRPVALALAVALILETRPTYRASPGLYSERLYSARGTYRTYRALAASPSERVALLYSGLYARGPHETHRILESERARGASPASNSERLYSASNTHRLEUPHELEUGLNMETASNSERLEUARGALAGLUASPTHRALAVALTYRTYRCYSALATHRASNASPASPTYRTRPGLYGLNGLYTHRLEUVALTHRVALSERSERASPLYSTHRHISTHRCYSPROPROCYSPROALAPROGLULEULEUGLYGLYPROSERVALPHELEUPHEPROPROLYSPROLYSASPTHRLEUMETILESERARGTHRPROGLUVALTHRCYSVALVALVALASPVALSERHISGLUASPPROGLUVALLYSPHEASNTRPTYRVALASPGLYVALGLUVALHISASNALALYSTHRLYSPROARGGLUGLUGLNTYRASNSERTHRTYRARGVALVALSERVALLEUTHRVALLEUHISGLNASPTRPLEUASNGLYLYSGLUTYRLYSCYSLYSVALSERASNLYSALALEUPROALAPROILEGLULYSTHRILESERLYSALALYSGLYGLNPROARGGLUPROGLNVALTYRTHRLEUPROPROSERARGASPGLULEUTHRLYSASNGLNVALSERLEUTHRCYSLEUVALLYSGLYPHETYRPROSERASPILEALAVALGLUTRPGLUSERASNGLYGLNPROGLUASNASNTYRLYSTHRTHRPROPROVALLEUASPSERASPGLYSERPHEPHELEUTYRSERLYSLEUTHRVALASPLYSSERARGTRPGLNGLNGLYASNVALPHESERCYSSERVALMETHISGLUALALEUHISASNHISTYRTHRGLNLYSSERLEUSERLEUSERPROGLYLYS

SEQ ID NO: 20 - protein, 1833 aa, Artificial sequence
GLUILEVALLEUTHRGLNSERPROALATHRLEUSERLEUSERPROGLYGLUARGALATHRLEUSERCYSARGALASERLYSGLYVALSERTHRSERGLYTYRSERTYRLEUHISTRPTYRGLNGLNLYSPROGLYGLNALAPROARGLEULEUILETYRLEUALASERTYRLEUGLUSERGLYVALPROALAARGPHESERGLYSERGLYSERGLYTHRASPPHETHRLEUTHRILESERSERLEUGLUPROGLUASPPHEALAVALTYRTYRCYSGLNHISSERARGASPLEUPROLEUTHRPHEGLYGLYGLYTHRLYSVALGLUILELYSGLYGLYGLYGLYSERGLYGLYGLYGLYSERGLYGLYGLYGLYSERGLNVALGLNLEUVALGLNSERGLYVALGLUVALLYSLYSPROGLYALASERVALLYSVALSERCYSLYSALASERGLYTYRTHRPHETHRASNTYRTYRMETTYRTRPVALARGGLNALAPROGLYGLNGLYLEUGLUTRPMETGLYGLYILEASNPROSERASNGLYGLYTHRASNPHEASNGLULYSPHELYSASNARGVALTHRLEUTHRTHRASPSERSERTHRTHRTHRALATYRMETGLULEULYSSERLEUGLNPHEASPASPTHRALAVALTYRTYRCYSALAARGARGASPTYRARGPHEASPMETGLYPHEASPTYRTRPGLYGLNGLYTHRTHRVALTHRVALSERSERASPLYSTHRHISTHRCYSPROPROCYSPROALAPROGLULEULEUGLYGLYPROSERVALPHELEUPHEPROPROLYSPROLYSASPTHRLEUMETILESERARGTHRPROGLUVALTHRCYSVALVALVALASPVALSERHISGLUASPPROGLUVALLYSPHEASNTRPTYRVALASPGLYVALGLUVALHISASNALALYSTHRLYSPROARGGLUGLUGLNTYRASNSERTHRTYRARGVALVALSERVALLEUTHRVALLEUHISGLNASPTRPLEUASNGLYLYSGLUTYRLYSCYSLYSVALSERASNLYSALALEUPROALAPROILEGLULYSTHRILESERLYSALALYSGLYGLNPROARGGLUPROGLNVALTYRTHRLEUPROPROSERARGASPGLULEUTHRLYSASNGLNVALSERLEUTHRCYSLEUVALLYSGLYPHETYRPROSERASPILEALAVALGLUTRPGLUSERASNGLYGLNPROGLUASNASNTYRLYSTHRTHRPROPROVALLEUASPSERASPGLYSERPHEPHELEUTYRSERLYSLEUTHRVALASPLYSSERARGTRPGLNGLNGLYASNVALPHESERCYSSERVALMETHISGLUALALEUHISASNHISTYRTHRGLNLYSSERLEUSERLEUSERPROGLYLYSGLYGLYGLYGLYSERALAPROTHRSERSERSERTHRLYSLYSTHRGLNLEUGLNLEUGLUHISLEULEULEUASPLEUGLNMETILELEUASNGLYILEASNASNTYRLYSASNPROLYSLEUTHRLEUMETLEUTHRALALYSPHETYRMETPROLYSLYSALATHRGLULEULYSHISLEUGLNCYSLEUGLUGLUGLULEULYSPROLEUGLUGLUVALLEUASNLEUALAGLNSERLYSASNPHEHISLEUARGPROARGASPLEUILESERASNILEASNVALILEVALLEUGLULEULYSGLYSERGLUTHRTHRPHEMETCYSGLUTYRALAASPGLUTHRALATHRILEVALGLUPHELEUASNARGTRPILETHRPHECYSGLNSERILEILESERTHRLEUTHR

SEQ ID NO: 21 - protein, 1833 aa, Artificial sequence
ALAPROTHRSERSERSERTHRLYSLYSTHRGLNLEUGLNLEUGLUHISLEULEULEUASPLEUGLNMETILELEUASNGLYILEASNASNTYRLYSASNPROLYSLEUTHRLEUMETLEUTHRALALYSPHETYRMETPROLYSLYSALATHRGLULEULYSHISLEUGLNCYSLEUGLUGLUGLULEULYSPROLEUGLUGLUVALLEUASNLEUALAGLNSERLYSASNPHEHISLEUARGPROARGASPLEUILESERASNILEASNVALILEVALLEUGLULEULYSGLYSERGLUTHRTHRPHEMETCYSGLUTYRALAASPGLUTHRALATHRILEVALGLUPHELEUASNARGTRPILETHRPHECYSGLNSERILEILESERTHRLEUTHRGLYGLYGLYGLYSERGLUILEVALLEUTHRGLNSERPROALATHRLEUSERLEUSERPROGLYGLUARGALATHRLEUSERCYSARGALASERLYSGLYVALSERTHRSERGLYTYRSERTYRLEUHISTRPTYRGLNGLNLYSPROGLYGLNALAPROARGLEULEUILETYRLEUALASERTYRLEUGLUSERGLYVALPROALAARGPHESERGLYSERGLYSERGLYTHRASPPHETHRLEUTHRILESERSERLEUGLUPROGLUASPPHEALAVALTYRTYRCYSGLNHISSERARGASPLEUPROLEUTHRPHEGLYGLYGLYTHRLYSVALGLUILELYSGLYGLYGLYGLYSERGLYGLYGLYGLYSERGLYGLYGLYGLYSERGLNVALGLNLEUVALGLNSERGLYVALGLUVALLYSLYSPROGLYALASERVALLYSVALSERCYSLYSALASERGLYTYRTHRPHETHRASNTYRTYRMETTYRTRPVALARGGLNALAPROGLYGLNGLYLEUGLUTRPMETGLYGLYILEASNPROSERASNGLYGLYTHRASNPHEASNGLULYSPHELYSASNARGVALTHRLEUTHRTHRASPSERSERTHRTHRTHRALATYRMETGLULEULYSSERLEUGLNPHEASPASPTHRALAVALTYRTYRCYSALAARGARGASPTYRARGPHEASPMETGLYPHEASPTYRTRPGLYGLNGLYTHRTHRVALTHRVALSERSERASPLYSTHRHISTHRCYSPROPROCYSPROALAPROGLULEULEUGLYGLYPROSERVALPHELEUPHEPROPROLYSPROLYSASPTHRLEUMETILESERARGTHRPROGLUVALTHRCYSVALVALVALASPVALSERHISGLUASPPROGLUVALLYSPHEASNTRPTYRVALASPGLYVALGLUVALHISASNALALYSTHRLYSPROARGGLUGLUGLNTYRASNSERTHRTYRARGVALVALSERVALLEUTHRVALLEUHISGLNASPTRPLEUASNGLYLYSGLUTYRLYSCYSLYSVALSERASNLYSALALEUPROALAPROILEGLULYSTHRILESERLYSALALYSGLYGLNPROARGGLUPROGLNVALTYRTHRLEUPROPROSERARGASPGLULEUTHRLYSASNGLNVALSERLEUTHRCYSLEUVALLYSGLYPHETYRPROSERASPILEALAVALGLUTRPGLUSERASNGLYGLNPROGLUASNASNTYRLYSTHRTHRPROPROVALLEUASPSERASPGLYSERPHEPHELEUTYRSERLYSLEUTHRVALASPLYSSERARGTRPGLNGLNGLYASNVALPHESERCYSSERVALMETHISGLUALALEUHISASNHISTYRTHRGLNLYSSERLEUSERLEUSERPROGLYLYS

SEQ ID NO: 22 - protein, 1419 aa, Artificial sequence
SERTYRGLULEUTHRGLNPROPROSERALASERVALASNVALGLYGLUTHRVALLYSILETHRCYSSERGLYASPGLNLEUPROLYSTYRPHEALAASPTRPPHEHISGLNARGSERASPGLNTHRILELEUGLNVALILETYRASPASPASNLYSARGPROSERGLYILEPROGLUARGILESERGLYSERSERSERGLYTHRTHRALATHRLEUTHRILEARGASPVALARGALAGLUASPGLUGLYASPTYRTYRCYSPHESERGLYTYRVALASPSERASPSERLYSLEUTYRVALPHEGLYSERGLYTHRGLNLEUTHRVALLEUGLYGLYGLYGLYSERGLYGLYGLYGLYSERGLYGLYGLYGLYSERGLUVALARGLEULEUGLUSERGLYGLYGLYLEUVALLYSPROGLUGLYSERLEULYSLEUSERCYSVALALASERGLYPHETHRPHESERASPTYRPHEMETSERTRPVALARGGLNALAPROGLYLYSGLYLEUGLUTRPVALALAHISILETYRTHRLYSSERTYRASNTYRALATHRTYRTYRSERGLYSERVALLYSGLYARGPHETHRILESERARGASPASPSERARGSERMETVALTYRLEUGLNMETASNASNLEUARGTHRGLUASPTHRALATHRTYRTYRCYSTHRARGASPGLYSERGLYTYRPROSERLEUASPPHETRPGLYGLNGLYTHRGLNVALTHRVALSERSERASPLYSTHRHISTHRCYSPROPROCYSPROALAPROGLULEULEUGLYGLYPROSERVALPHELEUPHEPROPROLYSPROLYSASPTHRLEUMETILESERARGTHRPROGLUVALTHRCYSVALVALVALASPVALSERHISGLUASPPROGLUVALLYSPHEASNTRPTYRVALASPGLYVALGLUVALHISASNALALYSTHRLYSPROARGGLUGLUGLNTYRASNSERTHRTYRARGVALVALSERVALLEUTHRVALLEUHISGLNASPTRPLEUASNGLYLYSGLUTYRLYSCYSLYSVALSERASNLYSALALEUPROALAPROILEGLULYSTHRILESERLYSALALYSGLYGLNPROARGGLUPROGLNVALTYRTHRLEUPROPROCYSARGASPGLULEUTHRLYSASNGLNVALSERLEUTRPCYSLEUVALLYSGLYPHETYRPROSERASPILEALAVALGLUTRPGLUSERASNGLYGLNPROGLUASNASNTYRLYSTHRTHRPROPROVALLEUASPSERASPGLYSERPHEPHELEUTYRSERALALEUTHRVALASPLYSSERARGTRPGLNGLNGLYASNVALPHESERCYSSERVALMETHISGLUALALEUHISASNHISTYRTHRGLNLYSSERLEUSERLEUSERPROGLYLYS

SEQ ID NO: 23 - protein, 1401 aa, Artificial sequence
ASPILEGLNMETTHRGLNSERPROSERSERLEUSERALASERVALGLYASPARGVALTHRILETHRCYSARGALASERGLNASPVALSERTHRALAVALALATRPTYRGLNGLNLYSPROGLYLYSALAPROLYSLEULEUILETYRSERALASERPHELEUTYRSERGLYVALPROSERARGPHESERGLYSERGLYSERGLYTHRASPPHETHRLEUTHRILESERSERLEUGLNPROGLUASPPHEALATHRTYRTYRCYSGLNGLNTYRLEUTYRHISPROALATHRPHEGLYGLNGLYTHRLYSVALGLUILELYSGLYGLYGLYGLYSERGLYGLYGLYGLYSERGLYGLYGLYGLYSERGLUVALGLNLEUVALGLUSERGLYGLYGLYLEUVALGLNPROGLYGLYSERLEUARGLEUSERCYSALAALASERGLYPHETHRPHESERASPSERTRPILEHISTRPVALARGGLNALAPROGLYLYSGLYLEUGLUTRPVALALATRPILESERPROTYRGLYGLYSERTHRTYRTYRALAASPSERVALLYSGLYARGPHETHRILESERALAASPTHRSERLYSASNTHRALATYRLEUGLNMETASNSERLEUARGALAGLUASPTHRALAVALTYRTYRCYSALAARGARGHISTRPPROGLYGLYPHEASPTYRTRPGLYGLNGLYTHRLEUVALTHRVALSERALAASPLYSTHRHISTHRCYSPROPROCYSPROALAPROGLULEULEUGLYGLYPROSERVALPHELEUPHEPROPROLYSPROLYSASPTHRLEUMETILESERARGTHRPROGLUVALTHRCYSVALVALVALASPVALSERHISGLUASPPROGLUVALLYSPHEASNTRPTYRVALASPGLYVALGLUVALHISASNALALYSTHRLYSPROARGGLUGLUGLNTYRASNSERTHRTYRARGVALVALSERVALLEUTHRVALLEUHISGLNASPTRPLEUASNGLYLYSGLUTYRLYSCYSLYSVALSERASNLYSALALEUPROALAPROILEGLULYSTHRILESERLYSALALYSGLYGLNPROARGGLUPROGLNVALTYRTHRLEUPROPROCYSARGASPGLULEUTHRLYSASNGLNVALSERLEUTRPCYSLEUVALLYSGLYPHETYRPROSERASPILEALAVALGLUTRPGLUSERASNGLYGLNPROGLUASNASNTYRLYSTHRTHRPROPROVALLEUASPSERASPGLYSERPHEPHELEUTYRSERALALEUTHRVALASPLYSSERARGTRPGLNGLNGLYASNVALPHESERCYSSERVALMETHISGLUALALEUHISASNHISTYRTHRGLNLYSSERLEUSERLEUSERPROGLYLYS